European Patent Application EP 4 744 671 A1, published May 20, 2026. Title: 聚乳酸及其共聚物在促进骨组织、软骨组织生长中的应用. Applicant: 长春圣博玛生物材料有限公司. The sequence listing filed with the application follows.

SEQUENCE LISTING (8 sequences)

SEQ ID NO: 1 - DNA, 20 bp, synthetic construct
  source 1..20: mol_type = other DNA
gagcttggaacggtacgata

SEQ ID NO: 2 - DNA, 24 bp, synthetic construct
  source 1..24: mol_type = other DNA
tgaaggtggagtagagcacagagc

SEQ ID NO: 3 - DNA, 21 bp, synthetic construct
  source 1..21: mol_type = other DNA
tgggaaagaagacttggctgg

SEQ ID NO: 4 - DNA, 23 bp, synthetic construct
  source 1..23: mol_type = other DNA
ctccaccaatgtagtatccacga

SEQ ID NO: 5 - DNA, 24 bp, synthetic construct
  source 1..24: mol_type = other DNA
tgggcagaggtataatgataagga

SEQ ID NO: 6 - DNA, 23 bp, synthetic construct
  source 1..23: mol_type = other DNA
cttcacagattatgtcgtcgcag

SEQ ID NO: 7 - DNA, 20 bp, synthetic construct
  source 1..20: mol_type = other DNA
tgctccccagttgtcttatg

SEQ ID NO: 8 - DNA, 20 bp, synthetic construct
  source 1..20: mol_type = other DNA
atcatctccgttcttgccag